European Patent Specification EP 3 128 008 B1, published May 29, 2024. Title: Novel Double Strand Oligo RNA and Pharmaceutical Compositions For Preventing or Treating Fibrosis or Respiratory Diseases Containing The Same. Applicant: Bioneer Corporation. The sequence listing filed with the application follows.

SEQUENCE LISTING (343 sequences)

SEQ ID NO: 1 - RNA, 19 nt, Artificial Sequence
  siRNA
ggaguaugauaaugaacca

SEQ ID NO: 2 - RNA, 19 nt, Artificial Sequence
  siRNA
caguaguagcugucacuau

SEQ ID NO: 3 - RNA, 19 nt, Artificial Sequence
  siRNA
agacucacagcgaggauga

SEQ ID NO: 4 - RNA, 19 nt, Artificial Sequence
  siRNA
cacaaauauccggcuauau

SEQ ID NO: 5 - RNA, 19 nt, Artificial Sequence
  siRNA
caccauaagcgaaaugccu

SEQ ID NO: 6 - RNA, 19 nt, Artificial Sequence
  siRNA
gauuacuuuggugaacggu

SEQ ID NO: 7 - RNA, 19 nt, Artificial Sequence
  siRNA
caguugucacuuuuuauga

SEQ ID NO: 8 - RNA, 19 nt, Artificial Sequence
  siRNA
ggaccuauccaagauugca

SEQ ID NO: 9 - RNA, 19 nt, Artificial Sequence
  siRNA
cguuaucacagugcaccuu

SEQ ID NO: 10 - RNA, 19 nt, Artificial Sequence
  siRNA
ccuagcugaggacaaugca

SEQ ID NO: 11 - RNA, 19 nt, Artificial Sequence
  siRNA
ccuagcugaggacaaugca

SEQ ID NO: 12 - RNA, 19 nt, Artificial Sequence
  siRNA
cucagaggaguaugauaau

SEQ ID NO: 13 - RNA, 19 nt, Artificial Sequence
  siRNA
cgguggacuugagcuuucu

SEQ ID NO: 14 - RNA, 19 nt, Artificial Sequence
  siRNA
gguggugacaugcaauugu

SEQ ID NO: 15 - RNA, 19 nt, Artificial Sequence
  siRNA
cagggaauaugaaggagaa

SEQ ID NO: 16 - RNA, 19 nt, Artificial Sequence
  siRNA
ggaggcuucgacaagaaaa

SEQ ID NO: 17 - RNA, 19 nt, Artificial Sequence
  siRNA
ccgguggaaccaaugagaa

SEQ ID NO: 18 - RNA, 19 nt, Artificial Sequence
  siRNA
ccggcuauauuauagauga

SEQ ID NO: 19 - RNA, 19 nt, Artificial Sequence
  siRNA
agaauccaugcacugccaa

SEQ ID NO: 20 - RNA, 19 nt, Artificial Sequence
  siRNA
caaggaccuauccaagauu

SEQ ID NO: 21 - RNA, 19 nt, Artificial Sequence
  siRNA
caaauauccggcuauauua

SEQ ID NO: 22 - RNA, 19 nt, Artificial Sequence
  siRNA
gggacuacgacuacucaga

SEQ ID NO: 23 - RNA, 19 nt, Artificial Sequence
  siRNA
gcgaaugcagauacaucga

SEQ ID NO: 24 - RNA, 19 nt, Artificial Sequence
  siRNA
gccacaccggaaaugacau

SEQ ID NO: 25 - RNA, 19 nt, Artificial Sequence
  siRNA
agaguugaacaggugauua

SEQ ID NO: 26 - RNA, 19 nt, Artificial Sequence
  siRNA
gaaccacaaauauccggcu

SEQ ID NO: 27 - RNA, 19 nt, Artificial Sequence
  siRNA
cauaagcgaaaugccuucu

SEQ ID NO: 28 - RNA, 19 nt, Artificial Sequence
  siRNA
guuuccaccauaagcgaaa

SEQ ID NO: 29 - RNA, 19 nt, Artificial Sequence
  siRNA
caggugauuaagcccaaga

SEQ ID NO: 30 - RNA, 19 nt, Artificial Sequence
  siRNA
ccacaccggaaaugacauu

SEQ ID NO: 31 - RNA, 19 nt, Artificial Sequence
  siRNA
gagtgaaatgccttctagt

SEQ ID NO: 32 - RNA, 19 nt, Artificial Sequence
  siRNA
cagagttgaacaggtagtt

SEQ ID NO: 33 - RNA, 19 nt, Artificial Sequence
  siRNA
ctggattggacctcaatga

SEQ ID NO: 34 - RNA, 19 nt, Artificial Sequence
  siRNA
gaaaactcacagcatgatt

SEQ ID NO: 35 - RNA, 19 nt, Artificial Sequence
  siRNA
gaaacttcgacaagagaat

SEQ ID NO: 36 - RNA, 19 nt, Artificial Sequence
  siRNA
caggaaatatgaaggagaa

SEQ ID NO: 37 - RNA, 19 nt, Artificial Sequence
  siRNA
gcaaatatatagagcacct

SEQ ID NO: 38 - RNA, 19 nt, Artificial Sequence
  siRNA
ggtgctgtcgctcttgata

SEQ ID NO: 39 - RNA, 19 nt, Artificial Sequence
  siRNA
tcagagttgaacaggtagt

SEQ ID NO: 40 - RNA, 19 nt, Artificial Sequence
  siRNA
gaaagaaacttcgacaaga

SEQ ID NO: 41 - RNA, 19 nt, Artificial Sequence
  siRNA
gacaatacgtcaggaaata

SEQ ID NO: 42 - RNA, 19 nt, Artificial Sequence
  siRNA
caggatatcacattggagt

SEQ ID NO: 43 - RNA, 19 nt, Artificial Sequence
  siRNA
ctctttccagtggatcata

SEQ ID NO: 44 - RNA, 19 nt, Artificial Sequence
  siRNA
cggctcaggccattatgct

SEQ ID NO: 45 - RNA, 19 nt, Artificial Sequence
  siRNA
ggaccacagtgctgatgga

SEQ ID NO: 46 - RNA, 19 nt, Artificial Sequence
  siRNA
gctgctggattggacctca

SEQ ID NO: 47 - RNA, 19 nt, Artificial Sequence
  siRNA
gttattacagtccagctta

SEQ ID NO: 48 - RNA, 19 nt, Artificial Sequence
  siRNA
tggacctcaatgacaccta

SEQ ID NO: 49 - RNA, 19 nt, Artificial Sequence
  siRNA
ctggctatattgtcgatga

SEQ ID NO: 50 - RNA, 19 nt, Artificial Sequence
  siRNA
gacggaaagtgaaaatact

SEQ ID NO: 51 - RNA, 19 nt, Artificial Sequence
  siRNA
gtatgataacgaaccacaa

SEQ ID NO: 52 - RNA, 19 nt, Artificial Sequence
  siRNA
acattggagtcactgccaa

SEQ ID NO: 53 - RNA, 19 nt, Artificial Sequence
  siRNA
ccaagtcatagccataaat

SEQ ID NO: 54 - RNA, 19 nt, Artificial Sequence
  siRNA
agtgaaatgccttctagta

SEQ ID NO: 55 - RNA, 19 nt, Artificial Sequence
  siRNA
gataacgaaccacaaatac

SEQ ID NO: 56 - RNA, 19 nt, Artificial Sequence
  siRNA
tgcattagcagccatagct

SEQ ID NO: 57 - RNA, 19 nt, Artificial Sequence
  siRNA
gcattcacggagaatgcaa

SEQ ID NO: 58 - RNA, 19 nt, Artificial Sequence
  siRNA
ggagtcactgccaagtcat

SEQ ID NO: 59 - RNA, 19 nt, Artificial Sequence
  siRNA
aggtgcacgaaggtaaaaa

SEQ ID NO: 60 - RNA, 19 nt, Artificial Sequence
  siRNA
cagcatgattgacagtagt

SEQ ID NO: 61 - RNA, 19 nt, Artificial Sequence
  siRNA
cttagaagacaatacgtca

SEQ ID NO: 62 - RNA, 19 nt, Artificial Sequence
  siRNA
agagttgaacaggtagtta

SEQ ID NO: 63 - RNA, 19 nt, Artificial Sequence
  siRNA
tgatgagtcggtcctcttt

SEQ ID NO: 64 - RNA, 19 nt, Artificial Sequence
  siRNA
atatatagagcacctggaa

SEQ ID NO: 65 - RNA, 19 nt, Artificial Sequence
  siRNA
gagttgaacaggtagttaa

SEQ ID NO: 66 - RNA, 19 nt, Artificial Sequence
  siRNA
cattcacggagaatgcaaa

SEQ ID NO: 67 - RNA, 19 nt, Artificial Sequence
  siRNA
ggaccctttttgttatgat

SEQ ID NO: 68 - RNA, 19 nt, Artificial Sequence
  siRNA
cagaagagtatgataacga

SEQ ID NO: 69 - RNA, 19 nt, Artificial Sequence
  siRNA
ccagtggatcataagacaa

SEQ ID NO: 70 - RNA, 19 nt, Artificial Sequence
  siRNA
gctgttattacagtccagc

SEQ ID NO: 71 - RNA, 19 nt, Artificial Sequence
  siRNA
gggaagcgtgaaccatttt

SEQ ID NO: 72 - RNA, 19 nt, Artificial Sequence
  siRNA
cacagtgctgatggatttg

SEQ ID NO: 73 - RNA, 19 nt, Artificial Sequence
  siRNA
agtcagagttgaacaggta

SEQ ID NO: 74 - RNA, 19 nt, Artificial Sequence
  siRNA
tggaagcagtaacatgcaa

SEQ ID NO: 75 - RNA, 19 nt, Artificial Sequence
  siRNA
cacgaaggtaaaaagtatt

SEQ ID NO: 76 - RNA, 19 nt, Artificial Sequence
  siRNA
agaagagtatgataacgaa

SEQ ID NO: 77 - RNA, 19 nt, Artificial Sequence
  siRNA
gaagcgtgaaccattttct

SEQ ID NO: 78 - RNA, 19 nt, Artificial Sequence
  siRNA
ggctatattgtcgatgatt

SEQ ID NO: 79 - RNA, 19 nt, Artificial Sequence
  siRNA
gagtcactgccaagtcata

SEQ ID NO: 80 - RNA, 19 nt, Artificial Sequence
  siRNA
caatggaccctttttgtta

SEQ ID NO: 81 - RNA, 19 nt, Artificial Sequence
  siRNA
gcacgaaggtaaaaagtat

SEQ ID NO: 82 - RNA, 19 nt, Artificial Sequence
  siRNA
tgaaatgccttctagtagt

SEQ ID NO: 83 - RNA, 19 nt, Artificial Sequence
  siRNA
tggatcataagacaatgga

SEQ ID NO: 84 - RNA, 19 nt, Artificial Sequence
  siRNA
gtgagtgaaatgccttcta

SEQ ID NO: 85 - RNA, 19 nt, Artificial Sequence
  siRNA
gacctcaatgacacctact

SEQ ID NO: 86 - RNA, 19 nt, Artificial Sequence
  siRNA
cctcaatgacacctactct

SEQ ID NO: 87 - RNA, 19 nt, Artificial Sequence
  siRNA
gctgatggatttgaggtta

SEQ ID NO: 88 - RNA, 19 nt, Artificial Sequence
  siRNA
ggaagcagtaacatgcaaa

SEQ ID NO: 89 - RNA, 19 nt, Artificial Sequence
  siRNA
cagtaacatgcaaatgtca

SEQ ID NO: 90 - RNA, 19 nt, Artificial Sequence
  siRNA
gctatagcataactgaaga

SEQ ID NO: 91 - RNA, 19 nt, Artificial Sequence
  siRNA
ggatatcacattggagtca

SEQ ID NO: 92 - RNA, 19 nt, Artificial Sequence
  siRNA
ccctttttgttatgatggt

SEQ ID NO: 93 - RNA, 19 nt, Artificial Sequence
  siRNA
gtatataaaggtgcacgaa

SEQ ID NO: 94 - RNA, 19 nt, Artificial Sequence
  siRNA
ggacctcaatgacacctac

SEQ ID NO: 95 - RNA, 19 nt, Artificial Sequence
  siRNA
gctcttgatactcggctca

SEQ ID NO: 96 - RNA, 19 nt, Artificial Sequence
  siRNA
tgctgctggattggacctc

SEQ ID NO: 97 - RNA, 19 nt, Artificial Sequence
  siRNA
gaaccacaaatacctggct

SEQ ID NO: 98 - RNA, 19 nt, Artificial Sequence
  siRNA
cggtcctctttccagtgga

SEQ ID NO: 99 - RNA, 19 nt, Artificial Sequence
  siRNA
ttccaacacccgctcgttt

SEQ ID NO: 100 - RNA, 19 nt, Artificial Sequence
  siRNA
agagcacctggaagcagta

SEQ ID NO: 101 - RNA, 19 nt, Artificial Sequence
  siRNA
tctttccagtggatcataa

SEQ ID NO: 102 - RNA, 19 nt, Artificial Sequence
  siRNA
cctttttgttatgatggtt

SEQ ID NO: 103 - RNA, 19 nt, Artificial Sequence
  siRNA
cacctggaagcagtaacat

SEQ ID NO: 104 - RNA, 19 nt, Artificial Sequence
  siRNA
ctgaggaacgaaagaaact

SEQ ID NO: 105 - RNA, 19 nt, Artificial Sequence
  siRNA
gtgaaatgccttctagtag

SEQ ID NO: 106 - RNA, 19 nt, Artificial Sequence
  siRNA
ctactctgggaagcgtgaa

SEQ ID NO: 107 - RNA, 19 nt, Artificial Sequence
  siRNA
ctgggaagcgtgaaccatt

SEQ ID NO: 108 - RNA, 19 nt, Artificial Sequence
  siRNA
actactcagaagagtatga

SEQ ID NO: 109 - RNA, 19 nt, Artificial Sequence
  siRNA
catgcaaatgtcagcaaga

SEQ ID NO: 110 - RNA, 19 nt, Artificial Sequence
  siRNA
tgaggttacctcaagaagt

SEQ ID NO: 111 - RNA, 19 nt, Artificial Sequence
  siRNA
actcggctcaggccattat

SEQ ID NO: 112 - RNA, 19 nt, Artificial Sequence
  siRNA
ttcacggagaatgcaaata

SEQ ID NO: 113 - RNA, 19 nt, Artificial Sequence
  siRNA
ctgctggattggacctcaa

SEQ ID NO: 114 - RNA, 19 nt, Artificial Sequence
  siRNA
tgattcagtcagagttgaa

SEQ ID NO: 115 - RNA, 19 nt, Artificial Sequence
  siRNA
tgccaagtcatagccataa

SEQ ID NO: 116 - RNA, 19 nt, Artificial Sequence
  siRNA
ctcaagaagtgagatgtct

SEQ ID NO: 117 - RNA, 19 nt, Artificial Sequence
  siRNA
gccaagtcatagccataaa

SEQ ID NO: 118 - RNA, 19 nt, Artificial Sequence
  siRNA
ctcagaagagtatgataac

SEQ ID NO: 119 - RNA, 19 nt, Artificial Sequence
  siRNA
ttctgcattcacggagaat

SEQ ID NO: 120 - RNA, 19 nt, Artificial Sequence
  siRNA
taagacaatggaccctttt

SEQ ID NO: 121 - RNA, 19 nt, Artificial Sequence
  siRNA
aggttacctcaagaagtga

SEQ ID NO: 122 - RNA, 19 nt, Artificial Sequence
  siRNA
aatgccttctagtagtgaa

SEQ ID NO: 123 - RNA, 19 nt, Artificial Sequence
  siRNA
atgattcagtcagagttga

SEQ ID NO: 124 - RNA, 19 nt, Artificial Sequence
  siRNA
aaacaagacggaaagtgaa

SEQ ID NO: 125 - RNA, 19 nt, Artificial Sequence
  siRNA
tttctgcattcacggagaa

SEQ ID NO: 126 - RNA, 19 nt, Artificial Sequence
  siRNA
caaatacctggctatattg

SEQ ID NO: 127 - RNA, 19 nt, Artificial Sequence
  siRNA
tcttccaacacccgctcgt

SEQ ID NO: 128 - RNA, 19 nt, Artificial Sequence
  siRNA
gaagcagtaacatgcaaat

SEQ ID NO: 129 - RNA, 19 nt, Artificial Sequence
  siRNA
gatgattcagtcagagttg

SEQ ID NO: 130 - RNA, 19 nt, Artificial Sequence
  siRNA
tgcattcacggagaatgca

SEQ ID NO: 131 - RNA, 19 nt, Artificial Sequence
  siRNA
ctcagtgaggactcctaca

SEQ ID NO: 132 - RNA, 19 nt, Artificial Sequence
  siRNA
cactacgagatagccaaca

SEQ ID NO: 133 - RNA, 19 nt, Artificial Sequence
  siRNA
cagtcttccactacgagat

SEQ ID NO: 134 - RNA, 19 nt, Artificial Sequence
  siRNA
agctcctgagagacaacct

SEQ ID NO: 135 - RNA, 19 nt, Artificial Sequence
  siRNA
tcagtcttccactacgaga

SEQ ID NO: 136 - RNA, 19 nt, Artificial Sequence
  siRNA
agagacaacctgacgctgt

SEQ ID NO: 137 - RNA, 19 nt, Artificial Sequence
  siRNA
ccgaacggtatgaagacat

SEQ ID NO: 138 - RNA, 19 nt, Artificial Sequence
  siRNA
ctgaacaggccgaacggta

SEQ ID NO: 139 - RNA, 19 nt, Artificial Sequence
  siRNA
ctcctgagagacaacctga

SEQ ID NO: 140 - RNA, 19 nt, Artificial Sequence
  siRNA
gacatggcagctttcatga

SEQ ID NO: 141 - RNA, 19 nt, Artificial Sequence
  siRNA
cgaacggtatgaagacatg

SEQ ID NO: 142 - RNA, 19 nt, Artificial Sequence
  siRNA
agtaccgggagaaggtaga

SEQ ID NO: 143 - RNA, 19 nt, Artificial Sequence
  siRNA
acttttcagtcttccacta

SEQ ID NO: 144 - RNA, 19 nt, Artificial Sequence
  siRNA
gcatcgagcagaagagcaa

SEQ ID NO: 145 - RNA, 19 nt, Artificial Sequence
  siRNA
gcgaaacctgctttccgta

SEQ ID NO: 146 - RNA, 19 nt, Artificial Sequence
  siRNA
gtgaaagagtaccgggaga

SEQ ID NO: 147 - RNA, 19 nt, Artificial Sequence
  siRNA
gcgatgacaagaagcgcat

SEQ ID NO: 148 - RNA, 19 nt, Artificial Sequence
  siRNA
agtcttccactacgagata

SEQ ID NO: 149 - RNA, 19 nt, Artificial Sequence
  siRNA
tcagtgaggactcctacaa

SEQ ID NO: 150 - RNA, 19 nt, Artificial Sequence
  siRNA
ggtagagaccgagctcaga

SEQ ID NO: 151 - RNA, 19 nt, Artificial Sequence
  siRNA
ccgaggtgaaagagtaccg

SEQ ID NO: 152 - RNA, 19 nt, Artificial Sequence
  siRNA
caggccgaacggtatgaag

SEQ ID NO: 153 - RNA, 19 nt, Artificial Sequence
  siRNA
cggtatgaagacatggcag

SEQ ID NO: 154 - RNA, 19 nt, Artificial Sequence
  siRNA
tgctggactcgcacctcat

SEQ ID NO: 155 - RNA, 19 nt, Artificial Sequence
  siRNA
aagaagcgcatcatcgatt

SEQ ID NO: 156 - RNA, 19 nt, Artificial Sequence
  siRNA
ctggactcgcacctcatca

SEQ ID NO: 157 - RNA, 19 nt, Artificial Sequence
  siRNA
ggactcgcacctcatcaaa

SEQ ID NO: 158 - RNA, 19 nt, Artificial Sequence
  siRNA
gaagcgcatcatcgattct

SEQ ID NO: 159 - RNA, 19 nt, Artificial Sequence
  siRNA
gtcttccactacgagatag

SEQ ID NO: 160 - RNA, 19 nt, Artificial Sequence
  siRNA
aaggtagagaccgagctca

SEQ ID NO: 161 - RNA, 19 nt, Artificial Sequence
  siRNA
agcgaaacctgctttccgt

SEQ ID NO: 162 - RNA, 19 nt, Artificial Sequence
  siRNA
gactactaccgctacctag

SEQ ID NO: 163 - RNA, 19 nt, Artificial Sequence
  siRNA
cagagagccgcgtcttcta

SEQ ID NO: 164 - RNA, 19 nt, Artificial Sequence
  siRNA
gatgacaagaagcgcatca

SEQ ID NO: 165 - RNA, 19 nt, Artificial Sequence
  siRNA
catcgagcagaagagcaac

SEQ ID NO: 166 - RNA, 19 nt, Artificial Sequence
  siRNA
tgcagctcctgagagacaa

SEQ ID NO: 167 - RNA, 19 nt, Artificial Sequence
  siRNA
acggtatgaagacatggca

SEQ ID NO: 168 - RNA, 19 nt, Artificial Sequence
  siRNA
tggactcgcacctcatcaa

SEQ ID NO: 169 - RNA, 19 nt, Artificial Sequence
  siRNA
ggcgatgacaagaagcgca

SEQ ID NO: 170 - RNA, 19 nt, Artificial Sequence
  siRNA
tgaacaggccgaacggtat

SEQ ID NO: 171 - RNA, 19 nt, Artificial Sequence
  siRNA
aggccgaacggtatgaaga

SEQ ID NO: 172 - RNA, 19 nt, Artificial Sequence
  siRNA
tcgagcagaagagcaacga

SEQ ID NO: 173 - RNA, 19 nt, Artificial Sequence
  siRNA
tccactacgagatagccaa

SEQ ID NO: 174 - RNA, 19 nt, Artificial Sequence
  siRNA
ggtgaaagagtaccgggag

SEQ ID NO: 175 - RNA, 19 nt, Artificial Sequence
  siRNA
gccgaacggtatgaagaca

SEQ ID NO: 176 - RNA, 19 nt, Artificial Sequence
  siRNA
aggagatgccgcctaccaa

SEQ ID NO: 177 - RNA, 19 nt, Artificial Sequence
  siRNA
ggagcgaaacctgctttcc

SEQ ID NO: 178 - RNA, 19 nt, Artificial Sequence
  siRNA
cagtgaggactcctacaag

SEQ ID NO: 179 - RNA, 19 nt, Artificial Sequence
  siRNA
agcgcatcatcgattctgc

SEQ ID NO: 180 - RNA, 19 nt, Artificial Sequence
  siRNA
catcatgcagctcctgaga

SEQ ID NO: 181 - RNA, 19 nt, Artificial Sequence
  siRNA
gccgcgtcttctacctgaa

SEQ ID NO: 182 - RNA, 19 nt, Artificial Sequence
  siRNA
gagacaacctgacgctgtg

SEQ ID NO: 183 - RNA, 19 nt, Artificial Sequence
  siRNA
cgatgacaagaagcgcatc

SEQ ID NO: 184 - RNA, 19 nt, Artificial Sequence
  siRNA
cttccactacgagatagcc

SEQ ID NO: 185 - RNA, 19 nt, Artificial Sequence
  siRNA
ccactacgagatagccaac

SEQ ID NO: 186 - RNA, 19 nt, Artificial Sequence
  siRNA
gctcctgagagacaacctg

SEQ ID NO: 187 - RNA, 19 nt, Artificial Sequence
  siRNA
atcatcgattctgcccggt

SEQ ID NO: 188 - RNA, 19 nt, Artificial Sequence
  siRNA
tgagagacaacctgacgct

SEQ ID NO: 189 - RNA, 19 nt, Artificial Sequence
  siRNA
agacatggcagctttcatg

SEQ ID NO: 190 - RNA, 19 nt, Artificial Sequence
  siRNA
tcttccactacgagatagc

SEQ ID NO: 191 - RNA, 19 nt, Artificial Sequence
  siRNA
gaacaggccgaacggtatg

SEQ ID NO: 192 - RNA, 19 nt, Artificial Sequence
  siRNA
atgcagctcctgagagaca

SEQ ID NO: 193 - RNA, 19 nt, Artificial Sequence
  siRNA
accgagctcagaggtgtgt

SEQ ID NO: 194 - RNA, 19 nt, Artificial Sequence
  siRNA
cctgagagacaacctgacg

SEQ ID NO: 195 - RNA, 19 nt, Artificial Sequence
  siRNA
cacaccctcagtgaggact

SEQ ID NO: 196 - RNA, 19 nt, Artificial Sequence
  siRNA
ttccactacgagatagcca

SEQ ID NO: 197 - RNA, 19 nt, Artificial Sequence
  siRNA
acatggcagctttcatgaa

SEQ ID NO: 198 - RNA, 19 nt, Artificial Sequence
  siRNA
tgacaagaagcgcatcatc

SEQ ID NO: 199 - RNA, 19 nt, Artificial Sequence
  siRNA
aaggagatgccgcctacca

SEQ ID NO: 200 - RNA, 19 nt, Artificial Sequence
  siRNA
cttttcagtcttccactac

SEQ ID NO: 201 - RNA, 19 nt, Artificial Sequence
  siRNA
tcctgagagacaacctgac

SEQ ID NO: 202 - RNA, 19 nt, Artificial Sequence
  siRNA
gcagctcctgagagacaac

SEQ ID NO: 203 - RNA, 19 nt, Artificial Sequence
  siRNA
agccgcgtcttctacctga

SEQ ID NO: 204 - RNA, 19 nt, Artificial Sequence
  siRNA
attctgcccggtcagccta

SEQ ID NO: 205 - RNA, 19 nt, Artificial Sequence
  siRNA
actcgcacctcatcaaagg

SEQ ID NO: 206 - RNA, 19 nt, Artificial Sequence
  siRNA
agaccgagctcagaggtgt

SEQ ID NO: 207 - RNA, 19 nt, Artificial Sequence
  siRNA
gactcgcacctcatcaaag

SEQ ID NO: 208 - RNA, 19 nt, Artificial Sequence
  siRNA
agaagcgcatcatcgattc

SEQ ID NO: 209 - RNA, 19 nt, Artificial Sequence
  siRNA
gggtgactactaccgctac

SEQ ID NO: 210 - RNA, 19 nt, Artificial Sequence
  siRNA
caagaccaccttcgacgag

SEQ ID NO: 211 - RNA, 19 nt, Artificial Sequence
  siRNA
ctacgagatagccaacagc

SEQ ID NO: 212 - RNA, 19 nt, Artificial Sequence
  siRNA
tttcagtcttccactacga

SEQ ID NO: 213 - RNA, 19 nt, Artificial Sequence
  siRNA
aggtgaaagagtaccggga

SEQ ID NO: 214 - RNA, 19 nt, Artificial Sequence
  siRNA
aagcgcatcatcgattctg

SEQ ID NO: 215 - RNA, 19 nt, Artificial Sequence
  siRNA
gcatcatcgattctgcccg

SEQ ID NO: 216 - RNA, 19 nt, Artificial Sequence
  siRNA
aacggtatgaagacatggc

SEQ ID NO: 217 - RNA, 19 nt, Artificial Sequence
  siRNA
atcgagcagaagagcaacg

SEQ ID NO: 218 - RNA, 19 nt, Artificial Sequence
  siRNA
actactaccgctacctagc

SEQ ID NO: 219 - RNA, 19 nt, Artificial Sequence
  siRNA
ttttcagtcttccactacg

SEQ ID NO: 220 - RNA, 19 nt, Artificial Sequence
  siRNA
acgagatagccaacagccc

SEQ ID NO: 221 - RNA, 19 nt, Artificial Sequence
  siRNA
actaccgctacctagccga

SEQ ID NO: 222 - RNA, 19 nt, Artificial Sequence
  siRNA
actacgagatagccaacag

SEQ ID NO: 223 - RNA, 19 nt, Artificial Sequence
  siRNA
cccgaggtgaaagagtacc

SEQ ID NO: 224 - RNA, 19 nt, Artificial Sequence
  siRNA
cagctcctgagagacaacc

SEQ ID NO: 225 - RNA, 19 nt, Artificial Sequence
  siRNA
catcgattctgcccggtca

SEQ ID NO: 226 - RNA, 19 nt, Artificial Sequence
  siRNA
gagagacaacctgacgctg

SEQ ID NO: 227 - RNA, 19 nt, Artificial Sequence
  siRNA
gcgcatcatcgattctgcc

SEQ ID NO: 228 - RNA, 19 nt, Artificial Sequence
  siRNA
gaaggtagagaccgagctc

SEQ ID NO: 229 - RNA, 19 nt, Artificial Sequence
  siRNA
tcatcgattctgcccggtc

SEQ ID NO: 230 - RNA, 19 nt, Artificial Sequence
  siRNA
gaacggtatgaagacatgg

SEQ ID NO: 231 - RNA, 19 nt, Artificial Sequence
  siRNA
cgtaggaattgaggagtgt

SEQ ID NO: 232 - RNA, 19 nt, Artificial Sequence
  siRNA
cactacgagatcgccaaca

SEQ ID NO: 233 - RNA, 19 nt, Artificial Sequence
  siRNA
gctgtccagtattgagcag

SEQ ID NO: 234 - RNA, 19 nt, Artificial Sequence
  siRNA
gaccatgtttcctctcaat

SEQ ID NO: 235 - RNA, 19 nt, Artificial Sequence
  siRNA
cgagacaacctgacactgt

SEQ ID NO: 236 - RNA, 19 nt, Artificial Sequence
  siRNA
cgtcttccactacgagatc

SEQ ID NO: 237 - RNA, 19 nt, Artificial Sequence
  siRNA
cctgcgaagagcgaaacct

SEQ ID NO: 238 - RNA, 19 nt, Artificial Sequence
  siRNA
gctgcctctgatcgtagga

SEQ ID NO: 239 - RNA, 19 nt, Artificial Sequence
  siRNA
ccaagaccactttcgacga

SEQ ID NO: 240 - RNA, 19 nt, Artificial Sequence
  siRNA
gtctgctgggtgtgaccat

SEQ ID NO: 241 - RNA, 19 nt, Artificial Sequence
  siRNA
ctctgatcgtaggaattga

SEQ ID NO: 242 - RNA, 19 nt, Artificial Sequence
  siRNA
gctgggtgtgaccatgttt

SEQ ID NO: 243 - RNA, 19 nt, Artificial Sequence
  siRNA
gctgggtgtgaccatgttt

SEQ ID NO: 244 - RNA, 19 nt, Artificial Sequence
  siRNA
cgacaagaagcgcatcatt

SEQ ID NO: 245 - RNA, 19 nt, Artificial Sequence
  siRNA
ctgccgagaggactagtat

SEQ ID NO: 246 - RNA, 19 nt, Artificial Sequence
  siRNA
gcctctgatcgtaggaatt

SEQ ID NO: 247 - RNA, 19 nt, Artificial Sequence
  siRNA
gcgctgttcttgctccaaa

SEQ ID NO: 248 - RNA, 19 nt, Artificial Sequence
  siRNA
ctgcctctgatcgtaggaa

SEQ ID NO: 249 - RNA, 19 nt, Artificial Sequence
  siRNA
gccctgaacttttccgtct

SEQ ID NO: 250 - RNA, 19 nt, Artificial Sequence
  siRNA
tgcctctgatcgtaggaat

SEQ ID NO: 251 - RNA, 19 nt, Artificial Sequence
  siRNA
tgaccatgtttcctctcaa

SEQ ID NO: 252 - RNA, 19 nt, Artificial Sequence
  siRNA
ccatgtttcctctcaataa

SEQ ID NO: 253 - RNA, 19 nt, Artificial Sequence
  siRNA
ggtgacgacaagaagcgca

SEQ ID NO: 254 - RNA, 19 nt, Artificial Sequence
  siRNA
acttttccgtcttccacta

SEQ ID NO: 255 - RNA, 19 nt, Artificial Sequence
  siRNA
tccgtcttccactacgaga

SEQ ID NO: 256 - RNA, 19 nt, Artificial Sequence
  siRNA
ctctcctgcgaagagcgaa

SEQ ID NO: 257 - RNA, 19 nt, Artificial Sequence
  siRNA
ccaggaccaggctacttct

SEQ ID NO: 258 - RNA, 19 nt, Artificial Sequence
  siRNA
cctgctgcctctgatcgta

SEQ ID NO: 259 - RNA, 19 nt, Artificial Sequence
  siRNA
ccgaacgctatgaggacat

SEQ ID NO: 260 - RNA, 19 nt, Artificial Sequence
  siRNA
ccctgaacttttccgtctt

SEQ ID NO: 261 - RNA, 19 nt, Artificial Sequence
  siRNA
ccgtcttccactacgagat

SEQ ID NO: 262 - RNA, 19 nt, Artificial Sequence
  siRNA
gagacaacctgacactgtg

SEQ ID NO: 263 - RNA, 19 nt, Artificial Sequence
  siRNA
gcatgtctgctgggtgtga

SEQ ID NO: 264 - RNA, 19 nt, Artificial Sequence
  siRNA
tggctgagaactggacagt

SEQ ID NO: 265 - RNA, 19 nt, Artificial Sequence
  siRNA
gccgaacgctatgaggaca

SEQ ID NO: 266 - RNA, 19 nt, Artificial Sequence
  siRNA
ctgtccagtattgagcaga

SEQ ID NO: 267 - RNA, 19 nt, Artificial Sequence
  siRNA
gtattgagcagaaaagcaa

SEQ ID NO: 268 - RNA, 19 nt, Artificial Sequence
  siRNA
cagctgttgagcgcaccta

SEQ ID NO: 269 - RNA, 19 nt, Artificial Sequence
  siRNA
gacaacctgacactgtgga

SEQ ID NO: 270 - RNA, 19 nt, Artificial Sequence
  siRNA
tggagagagccagtctgat

SEQ ID NO: 271 - RNA, 19 nt, Artificial Sequence
  siRNA
cgaacgctatgaggacatg

SEQ ID NO: 272 - RNA, 19 nt, Artificial Sequence
  siRNA
ggtgctgtccagtattgag

SEQ ID NO: 273 - RNA, 19 nt, Artificial Sequence
  siRNA
gaagcgcatcattgactca

SEQ ID NO: 274 - RNA, 19 nt, Artificial Sequence
  siRNA
tcgtaggaattgaggagtg

SEQ ID NO: 275 - RNA, 19 nt, Artificial Sequence
  siRNA
gctgcgagacaacctgaca

SEQ ID NO: 276 - RNA, 19 nt, Artificial Sequence
  siRNA
tgctgtccagtattgagca

SEQ ID NO: 277 - RNA, 19 nt, Artificial Sequence
  siRNA
ctgttcttgctccaaaggg

SEQ ID NO: 278 - RNA, 19 nt, Artificial Sequence
  siRNA
cctctgatcgtaggaattg

SEQ ID NO: 279 - RNA, 19 nt, Artificial Sequence
  siRNA
ccaccggtgacgacaagaa

SEQ ID NO: 280 - RNA, 19 nt, Artificial Sequence
  siRNA
gtcttccactacgagatcg

SEQ ID NO: 281 - RNA, 19 nt, Artificial Sequence
  siRNA
ctacctgaagatgaagggt

SEQ ID NO: 282 - RNA, 19 nt, Artificial Sequence
  siRNA
ctataagaacgtggtgggc

SEQ ID NO: 283 - RNA, 19 nt, Artificial Sequence
  siRNA
ctctggccaagaccacttt

SEQ ID NO: 284 - RNA, 19 nt, Artificial Sequence
  siRNA
cgctgttcttgctccaaag

SEQ ID NO: 285 - RNA, 19 nt, Artificial Sequence
  siRNA
ccactttcgacgaggccat

SEQ ID NO: 286 - RNA, 19 nt, Artificial Sequence
  siRNA
tgagaactggacagtggca

SEQ ID NO: 287 - RNA, 19 nt, Artificial Sequence
  siRNA
ctggccaagaccactttcg

SEQ ID NO: 288 - RNA, 19 nt, Artificial Sequence
  siRNA
ttgagcagaaaagcaacga

SEQ ID NO: 289 - RNA, 19 nt, Artificial Sequence
  siRNA
tgcgagacaacctgacact

SEQ ID NO: 290 - RNA, 19 nt, Artificial Sequence
  siRNA
agctgttgagcgcacctaa

SEQ ID NO: 291 - RNA, 19 nt, Artificial Sequence
  siRNA
gaacttttccgtcttccac

SEQ ID NO: 292 - RNA, 19 nt, Artificial Sequence
  siRNA
aaaagcaacgaggagggct

SEQ ID NO: 293 - RNA, 19 nt, Artificial Sequence
  siRNA
tctcctgcgaagagcgaaa

SEQ ID NO: 294 - RNA, 19 nt, Artificial Sequence
  siRNA
ctgttgagcgcacctaacc

SEQ ID NO: 295 - RNA, 19 nt, Artificial Sequence
  siRNA
cctgaacttttccgtcttc

SEQ ID NO: 296 - RNA, 19 nt, Artificial Sequence
  siRNA
gctgttcttgctccaaagg

SEQ ID NO: 297 - RNA, 19 nt, Artificial Sequence
  siRNA
aggccgaacgctatgagga

SEQ ID NO: 298 - RNA, 19 nt, Artificial Sequence
  siRNA
attgaggagtgtcccgcct

SEQ ID NO: 299 - RNA, 19 nt, Artificial Sequence
  siRNA
gtgaccatgtttcctctca

SEQ ID NO: 300 - RNA, 19 nt, Artificial Sequence
  siRNA
caagaccactttcgacgag

SEQ ID NO: 301 - RNA, 19 nt, Artificial Sequence
  siRNA
aacttttccgtcttccact

SEQ ID NO: 302 - RNA, 19 nt, Artificial Sequence
  siRNA
tgatcgtaggaattgagga

SEQ ID NO: 303 - RNA, 19 nt, Artificial Sequence
  siRNA
ggagagagccagtctgatc

SEQ ID NO: 304 - RNA, 19 nt, Artificial Sequence
  siRNA
agcaggccgaacgctatga

SEQ ID NO: 305 - RNA, 19 nt, Artificial Sequence
  siRNA
aggacatggcagccttcat

SEQ ID NO: 306 - RNA, 19 nt, Artificial Sequence
  siRNA
acgacaagaagcgcatcat

SEQ ID NO: 307 - RNA, 19 nt, Artificial Sequence
  siRNA
accatgtttcctctcaata

SEQ ID NO: 308 - RNA, 19 nt, Artificial Sequence
  siRNA
tgccgagaggactagtatg

SEQ ID NO: 309 - RNA, 19 nt, Artificial Sequence
  siRNA
tctgatcgtaggaattgag

SEQ ID NO: 310 - RNA, 19 nt, Artificial Sequence
  siRNA
tgggtgtgaccatgtttcc

SEQ ID NO: 311 - RNA, 19 nt, Artificial Sequence
  siRNA
tgaacttttccgtcttcca

SEQ ID NO: 312 - RNA, 19 nt, Artificial Sequence
  siRNA
gaattgaggagtgtcccgc

SEQ ID NO: 313 - RNA, 19 nt, Artificial Sequence
  siRNA
tttccgtcttccactacga

SEQ ID NO: 314 - RNA, 19 nt, Artificial Sequence
  siRNA
ctgctgcctctgatcgtag

SEQ ID NO: 315 - RNA, 19 nt, Artificial Sequence
  siRNA
ggccctgaacttttccgtc

SEQ ID NO: 316 - RNA, 19 nt, Artificial Sequence
  siRNA
gccaagaccactttcgacg

SEQ ID NO: 317 - RNA, 19 nt, Artificial Sequence
  siRNA
tctggccaagaccactttc

SEQ ID NO: 318 - RNA, 19 nt, Artificial Sequence
  siRNA
ctgaacttttccgtcttcc

SEQ ID NO: 319 - RNA, 19 nt, Artificial Sequence
  siRNA
aagcgcatcattgactcag

SEQ ID NO: 320 - RNA, 19 nt, Artificial Sequence
  siRNA
tgttgagcgcacctaacca

SEQ ID NO: 321 - RNA, 19 nt, Artificial Sequence
  siRNA
tacctgaagatgaagggtg

SEQ ID NO: 322 - RNA, 19 nt, Artificial Sequence
  siRNA
accactttcgacgaggcca

SEQ ID NO: 323 - RNA, 19 nt, Artificial Sequence
  siRNA
acgaggccatggctgatct

SEQ ID NO: 324 - RNA, 19 nt, Artificial Sequence
  siRNA
gatcccactcttcttgcag

SEQ ID NO: 325 - RNA, 19 nt, Artificial Sequence
  siRNA
cttttccgtcttccactac

SEQ ID NO: 326 - RNA, 19 nt, Artificial Sequence
  siRNA
gccgagaggactagtatgg

SEQ ID NO: 327 - RNA, 19 nt, Artificial Sequence
  siRNA
gctgttgagcgcacctaac

SEQ ID NO: 328 - RNA, 19 nt, Artificial Sequence
  siRNA
caggaccaggctacttctc

SEQ ID NO: 329 - RNA, 19 nt, Artificial Sequence
  siRNA
cctataagaacgtggtggg

SEQ ID NO: 330 - RNA, 19 nt, Artificial Sequence
  siRNA
ctgggtgtgaccatgtttc

SEQ ID NO: 331 - RNA, 19 nt, Artificial Sequence
  siCONT
cuuacgcugaguacuucga

SEQ ID NO: 332 - RNA, 21 nt, Artificial Sequence
  mRPL13A-F
cgatagtgcatcttggccttt

SEQ ID NO: 333 - RNA, 21 nt, Artificial Sequence
  mRPL13A-R
cctgctgctctcaaggttgtt

SEQ ID NO: 334 - RNA, 20 nt, Artificial Sequence
  hRPL13A-F
agctcatgaggctacggaaa

SEQ ID NO: 335 - RNA, 19 nt, Artificial Sequence
  hRPL13A-R
cgtacattccagggcaaca

SEQ ID NO: 336 - RNA, 21 nt, Artificial Sequence
  mAR-F
ggtcttaggctcaggccatta

SEQ ID NO: 337 - RNA, 20 nt, Artificial Sequence
  mAR-R
cgcttatggtggaaacctct

SEQ ID NO: 338 - RNA, 20 nt, Artificial Sequence
  hAR-F
acacctactctgggaagcgt

SEQ ID NO: 339 - RNA, 20 nt, Artificial Sequence
  hAR-R
gccaggtatttgtggttcgt

SEQ ID NO: 340 - RNA, 19 nt, Artificial Sequence
  mSFN-F
gtgtgtgcgacaccgtact

SEQ ID NO: 341 - RNA, 19 nt, Artificial Sequence
  mSFN-R
ctcggctaggtagcggtag

SEQ ID NO: 342 - RNA, 21 nt, Artificial Sequence
  hSFN-F
agaagcgcatcattgactcag

SEQ ID NO: 343 - RNA, 21 nt, Artificial Sequence
  hSFN-R
tctcgtagtggaagacggaaa